European Patent Application EP 4 324 854 A1, published February 21, 2024. Title: USE OF ANTIBODY IN ANTI-TUMOR TREATMENT. Applicant: AKESO PHARMACEUTICALS, INC. AD Pharmaceuticals CO., LTD. Application EP22787605.9. The sequence listing filed with the application follows.

SEQUENCE LISTING (72 sequences)

SEQ ID NO: 1 - DNA, 372 bp, Artificial Sequence
  Artificial Sequence-nucleic acid sequence of heavy chain variable region of 4G10
caggtcaagctgcaggagtctggacctgagctggtgaagcctggagcttcaatgaagatatcctgcaaggcttctggttactcattcactggctacaccatgaactgggtgaagcagagccatggaaagaaccttgaatggattggacttattaatccttacaataatattactaactacaaccagaagttcatgggcaaggccacatttactgtagacaagtcatccagcacagcctacatggaactcctcagactgacatctgaagactctggagtctatttctgtgcaagactcgactataggtcttattggggccaagggactctggtcactgtctctgcagccaaaacgacacccccatctgtctat

SEQ ID NO: 2 - protein, 124 aa, Artificial Sequence
  Artificial Sequence-amino acid sequence of heavy chain variable region of 4G10
QVKLQESGPELVKPGASMKISCKASGYSFTGYTMNWVKQSHGKNLEWIGLINPYNNITNYNQKFMGKATFTVDKSSSTAYMELLRLTSEDSGVYFCARLDYRSYWGQGTLVTVSAAKTTPPSVY

SEQ ID NO: 3 - DNA, 378 bp, Artificial Sequence
  Artificial Sequence-nucleic acid sequence of light chain variable region of 4G10
caggctgttgtgactcaggaatctgcactcaccacatcacctggtgaaacagtcacactcacttgtcgctcaagtactggggctgttacaactagtaactttgccaactgggtccaagaaaaaccagatcatttattcactagtctaataggtggtaccaacaaccgagctccaggtgttcctgccagattctcaggctccctgattggagacaaggctgccctcaccatcacaggggcacagactgaggatgaggcaatatatttctgtgctctatggtacagcaaccattgggtgttcggtggaggaaccaaactgactgtcctaggccagcccaagtcttcgccatcagtcaccctgtttcaagggcaattctgc

SEQ ID NO: 4 - protein, 126 aa, Artificial Sequence
  Artificial Sequence-amino acid sequence of light chain variable region of 4G10
QAVVTQESALTTSPGETVTLTCRSSTGAVTTSNFANWVQEKPDHLFTSLIGGTNNRAPGVPARFSGSLIGDKAALTITGAQTEDEAIYFCALWYSNHWVFGGGTKLTVLGQPKSSPSVTLFQGQFC

SEQ ID NO: 5 - DNA, 345 bp, Artificial Sequence
  Artificial Sequence-nucleic acid sequence of heavy chain variable region of 4G10H1L1
caggtgcagctggtggagtctggggccgagctggtgaagcccggcgcctccatgaagatctcttgcaaggccagcggatacagtttcactggctataccatgaactgggtcaaacaggctccaggacagggactggagtggatcgggctgattaatccttacaacaacatcaccaactacaaccagaagttcatgggaaaagcaacctttacagtggacaagagcatttccacagcctacatggaactgagccggctgacttcagacgatagcggggtctatttttgtgcaaggctggattatcgctcttactgggggcagggaactctggtcactgtctccgct

SEQ ID NO: 6 - protein, 115 aa, Artificial Sequence
  Artificial Sequence-amino acid sequence of heavy chain variable region of 4G10H1L1
QVQLVESGAELVKPGASMKISCKASGYSFTGYTMNWVKQAPGQGLEWIGLINPYNNITNYNQKFMGKATFTVDKSISTAYMELSRLTSDDSGVYFCARLDYRSYWGQGTLVTVSA

SEQ ID NO: 7 - DNA, 327 bp, Artificial Sequence
  Artificial Sequence-nucleic acid sequence of light chain variable region of 4G10H1L1
caggctgtcgtcactcaggaaccttcactgactgtgagcccaggaggaactgtcaccctgacatgcggaagctccaccggagcagtgaccacatccaacttcgccaattgggtccaggaaaagccaggccaggcatttcgatccctgatcggaggcacaaacaatcgggcttcttgggtgcccgcaagattctcaggaagcctgctggggggaaaagccgctctgaccattagtggcgctcagcctgaggacgaagccgagtacttctgcgctctgtggtatagcaaccactgggtgtttggcgggggaacaaagctgactgtgctg

SEQ ID NO: 8 - protein, 109 aa, Artificial Sequence
  Artificial Sequence-amino acid sequence of light chain variable region of 4G10H1L1
QAVVTQEPSLTVSPGGTVTLTCGSSTGAVTTSNFANWVQEKPGQAFRSLIGGTNNRASWVPARFSGSLLGGKAALTISGAQPEDEAEYFCALWYSNHWVFGGGTKLTVL

SEQ ID NO: 9 - DNA, 345 bp, Artificial Sequence
  Artificial Sequence-nucleic acid sequence of heavy chain variable region of 4G10H3L3
caggtgcagctggtcgagtctggggccgaagtgaagaaacccggcgcctcagtgaaggtcagctgcaaggccagcgggtacagtttcactggatataccatgaactgggtccgacaggcccctggccaggggctggagtggatcggcctgattaacccttacaacaacatcactaactacgcacagaagttccaggggagagtgacctttacagtggacaccagcatttccacagcctacatggaactgtcccggctgagatctgacgatacaggcgtgtacttctgcgctaggctggattaccgcagctattggggacagggcacactggtgactgtcagcgca

SEQ ID NO: 10 - protein, 115 aa, Artificial Sequence
  Artificial Sequence-amino acid sequence of heavy chain variable region of 4G10H3L3
QVQLVESGAEVKKPGASVKVSCKASGYSFTGYTMNWVRQAPGQGLEWIGLINPYNNITNYAQKFQGRVTFTVDTSISTAYMELSRLRSDDTGVYFCARLDYRSYWGQGTLVTVSA

SEQ ID NO: 11 - DNA, 327 bp, Artificial Sequence
  Artificial Sequence-nucleic acid sequence of light chain variable region of 4G10H3L3
caggctgtcgtcactcaggaaccttcactgaccgtgtctcctggcgggactgtcaccctgacatgcggcagctccacaggggccgtgaccacaagtaacttcccaaattgggtccagcagaagccaggacaggctccccggagtctgatcggaggcaccaacaacaaggccagctggacacccgcacggttcagcggcagcctgctgggcggcaaggccgctctgacaattagcggagcccagcctgaggacgaagccgagtactattgcgctctgtggtactccaaccactgggtgttcggcggcggcaccaagctgactgtgctg

SEQ ID NO: 12 - protein, 109 aa, Artificial Sequence
  Artificial Sequence-amino acid sequence of light chain variable region of 4G10H3L3
QAVVTQEPSLTVSPGGTVTLTCGSSTGAVTTSNFPNWVQQKPGQAPRSLIGGTNNKASWTPARFSGSLLGGKAALTISGAQPEDEAEYYCALWYSNHWVFGGGTKLTVL

SEQ ID NO: 13 - DNA, 354 bp, Artificial Sequence
  Artificial Sequence-nucleic acid sequence of heavy chain variable region of 14C12
gaggtcaaactggtggagagcggcggcgggctggtgaagcccggcgggtcactgaaactgagctgcgccgcttccggcttcgcctttagctcctacgacatgtcatgggtgaggcagacccctgagaagcgcctggaatgggtcgctactatcagcggaggcgggcgatacacctactatcctgactctgtcaaagggagattcacaattagtcgggataacgccagaaatactctgtatctgcagatgtctagtctgcggtccgaggatacagctctgtactattgtgcaaaccggtacggcgaagcatggtttgcctattggggacagggcaccctggtgacagtctctgcc

SEQ ID NO: 14 - protein, 118 aa, Artificial Sequence
  Artificial Sequence-amino acid sequence of heavy chain variable region of 14C12
EVKLVESGGGLVKPGGSLKLSCAASGFAFSSYDMSWVRQTPEKRLEWVATISGGGRYTYYPDSVKGRFTISRDNARNTLYLQMSSLRSEDTALYYCANRYGEAWFAYWGQGTLVTVSA

SEQ ID NO: 15 - DNA, 321 bp, Artificial Sequence
  Artificial Sequence-nucleic acid sequence of light chain variable region of 14C12
gacattaagatgacacagtccccttcctcaatgtacgctagcctgggcgagcgagtgaccttcacatgcaaagcatcccaggacatcaacacatacctgtcttggtttcagcagaagccaggcaaaagccccaagaccctgatctaccgggccaatagactggtggacggggtccccagcagattctccggatctggcagtgggcaggattactccctgaccatcagctccctggagtatgaagacatgggcatctactattgcctgcagtatgatgagttccctctgacctttggagcaggcacaaaactggaactgaag

SEQ ID NO: 16 - protein, 107 aa, Artificial Sequence
  Artificial Sequence-amino acid sequence of light chain variable region of 14C12
DIKMTQSPSSMYASLGERVTFTCKASQDINTYLSWFQQKPGKSPKTLIYRANRLVDGVPSRFSGSGSGQDYSLTISSLEYEDMGIYYCLQYDEFPLTFGAGTKLELK

SEQ ID NO: 17 - DNA, 354 bp, Artificial Sequence
  Artificial Sequence-nucleic acid sequence of heavy chain variable region of 14C12H1L1
gaagtgcagctggtcgagtctgggggagggctggtgcagcccggcgggtcactgcgactgagctgcgcagcttccggattcgcctttagctcctacgacatgtcctgggtgcgacaggcaccaggaaagggactggattgggtcgctactatctcaggaggcgggagatacacctactatcctgacagcgtcaagggccggttcacaatctctagagataacagtaagaacaatctgtatctgcagatgaacagcctgagggctgaggacaccgcactgtactattgtgccaaccgctacggggaagcatggtttgcctattgggggcagggaaccctggtgacagtctctagt

SEQ ID NO: 18 - protein, 118 aa, Artificial Sequence
  Artificial Sequence-amino acid sequence of heavy chain variable region of 14C12H1L1
EVQLVESGGGLVQPGGSLRLSCAASGFAFSSYDMSWVRQAPGKGLDWVATISGGGRYTYYPDSVKGRFTISRDNSKNNLYLQMNSLRAEDTALYYCANRYGEAWFAYWGQGTLVTVSS

SEQ ID NO: 19 - DNA, 321 bp, Artificial Sequence
  Artificial Sequence-nucleic acid sequence of light chain variable region of 14C12H1L1
gacattcagatgactcagagcccctcctccatgtccgcctctgtgggcgacagggtcaccttcacatgccgcgctagtcaggatatcaacacctacctgagctggtttcagcagaagccagggaaaagccccaagacactgatctaccgggctaatagactggtgtctggagtcccaagtcggttcagtggctcagggagcggacaggactacactctgaccatcagctccctgcagcctgaggacatggcaacctactattgcctgcagtatgatgagttcccactgacctttggcgccgggacaaaactggagctgaag

SEQ ID NO: 20 - protein, 107 aa, Artificial Sequence
  Artificial Sequence-amino acid sequence of light chain variable region of 14C12H1L1
DIQMTQSPSSMSASVGDRVTFTCRASQDINTYLSWFQQKPGKSPKTLIYRANRLVSGVPSRFSGSGSGQDYTLTISSLQPEDMATYYCLQYDEFPLTFGAGTKLELK

SEQ ID NO: 21 - DNA, 1344 bp, Artificial Sequence
  Artificial Sequence-DNA sequence of 14C12H1L1 heavy chain (14C12H1)
gaagtgcagctggtcgagtctgggggagggctggtgcagcccggcgggtcactgcgactgagctgcgcagcttccggattcgcctttagctcctacgacatgtcctgggtgcgacaggcaccaggaaagggactggattgggtcgctactatctcaggaggcgggagatacacctactatcctgacagcgtcaagggccggttcacaatctctagagataacagtaagaacaatctgtatctgcagatgaacagcctgagggctgaggacaccgcactgtactattgtgccaaccgctacggggaagcatggtttgcctattgggggcagggaaccctggtgacagtctctagtgccagcaccaaaggacctagcgtgtttcctctcgccccctcctccaaaagcaccagcggaggaaccgctgctctcggatgtctggtgaaggactacttccctgaacccgtcaccgtgagctggaatagcggcgctctgacaagcggagtccatacattccctgctgtgctgcaaagcagcggactctattccctgtccagcgtcgtcacagtgcccagcagcagcctgggcacccagacctacatctgtaacgtcaaccacaagccctccaacaccaaggtggacaagaaagtggagcccaaatcctgcgacaagacacacacctgtcccccctgtcctgctcccgaactcctcggaggccctagcgtcttcctctttcctcccaaacccaaggacaccctcatgatcagcagaacccctgaagtcacctgtgtcgtcgtggatgtcagccatgaggaccccgaggtgaaattcaactggtatgtcgatggcgtcgaggtgcacaacgccaaaaccaagcccagggaggaacagtacaactccacctacagggtggtgtccgtgctgacagtcctccaccaggactggctgaacggcaaggagtacaagtgcaaggtgtccaacaaggctctccctgcccccattgagaagaccatcagcaaggccaaaggccaacccagggagccccaggtctatacactgcctccctccagggacgaactcaccaagaaccaggtgtccctgacctgcctggtcaagggcttttatcccagcgacatcgccgtcgagtgggagtccaacggacagcccgagaataactacaagaccacccctcctgtcctcgactccgacggctccttcttcctgtacagcaagctgaccgtggacaaaagcaggtggcagcagggaaacgtgttctcctgcagcgtgatgcacgaagccctccacaaccactacacccagaaaagcctgtccctgagccccggcaaa

SEQ ID NO: 22 - protein, 448 aa, Artificial Sequence
  Artificial Sequence-encoded amino acid sequence of 14C12H1L1 heavy chain (14C12H1)
EVQLVESGGGLVQPGGSLRLSCAASGFAFSSYDMSWVRQAPGKGLDWVATISGGGRYTYYPDSVKGRFTISRDNSKNNLYLQMNSLRAEDTALYYCANRYGEAWFAYWGQGTLVTVSSASTKGPSVFPLAPSSKSTSGGTAALGCLVKDYFPEPVTVSWNSGALTSGVHTFPAVLQSSGLYSLSSVVTVPSSSLGTQTYICNVNHKPSNTKVDKKVEPKSCDKTHTCPPCPAPELLGGPSVFLFPPKPKDTLMISRTPEVTCVVVDVSHEDPEVKFNWYVDGVEVHNAKTKPREEQYNSTYRVVSVLTVLHQDWLNGKEYKCKVSNKALPAPIEKTISKAKGQPREPQVYTLPPSRDELTKNQVSLTCLVKGFYPSDIAVEWESNGQPENNYKTTPPVLDSDGSFFLYSKLTVDKSRWQQGNVFSCSVMHEALHNHYTQKSLSLSPGK

SEQ ID NO: 23 - DNA, 642 bp, Artificial Sequence
  Artificial Sequence-DNA sequence of 14C12H1L1 light chain (14C12L1)
gacattcagatgactcagagcccctcctccatgtccgcctctgtgggcgacagggtcaccttcacatgccgcgctagtcaggatatcaacacctacctgagctggtttcagcagaagccagggaaaagccccaagacactgatctaccgggctaatagactggtgtctggagtcccaagtcggttcagtggctcagggagcggacaggactacactctgaccatcagctccctgcagcctgaggacatggcaacctactattgcctgcagtatgatgagttcccactgacctttggcgccgggacaaaactggagctgaagcgaactgtggccgctccctccgtcttcatttttcccccttctgacgaacagctgaaatcaggcacagccagcgtggtctgtctgctgaacaatttctaccctagagaggcaaaagtgcagtggaaggtcgataacgccctgcagtccggcaacagccaggagagtgtgactgaacaggactcaaaagatagcacctattccctgtctagtacactgactctgtccaaggctgattacgagaagcacaaagtgtatgcatgcgaagtgacacatcagggactgtcaagccccgtgactaagtcttttaaccggggcgaatgt

SEQ ID NO: 24 - protein, 214 aa, Artificial Sequence
  Artificial Sequence-encoded amino acid sequence of 14C12H1L1 light chain (14C12L1)
DIQMTQSPSSMSASVGDRVTFTCRASQDINTYLSWFQQKPGKSPKTLIYRANRLVSGVPSRFSGSGSGQDYTLTISSLQPEDMATYYCLQYDEFPLTFGAGTKLELKRTVAAPSVFIFPPSDEQLKSGTASVVCLLNNFYPREAKVQWKVDNALQSGNSQESVTEQDSKDSTYSLSSTLTLSKADYEKHKVYACEVTHQGLSSPVTKSFNRGEC

SEQ ID NO: 25 - protein, 15 aa, Artificial Sequence
  Artificial Sequence-amino acid sequence of Linker1
GGGGSGGGGSGGGGS

SEQ ID NO: 26 - protein, 20 aa, Artificial Sequence
  Artificial Sequence-amino acid sequence of Linker2
GGGGSGGGGSGGGGSGGGGS

SEQ ID NO: 27 - protein, 8 aa, Artificial Sequence
  Artificial Sequence-HCDR1 of 14C12
GFAFSSYD

SEQ ID NO: 28 - protein, 8 aa, Artificial Sequence
  Artificial Sequence-HCDR2 of 14C12
ISGGGRYT

SEQ ID NO: 29 - protein, 11 aa, Artificial Sequence
  Artificial Sequence-HCDR2 of 14C12
ANRYGEAWFAY

SEQ ID NO: 30 - protein, 6 aa, Artificial Sequence
  Artificial Sequence-LCDR1 of 14C12
QDINTY

SEQ ID NO: 31 - protein, 3 aa, Artificial Sequence
  Artificial Sequence-LCDR2 of 14C12
RAN

SEQ ID NO: 32 - protein, 9 aa, Artificial Sequence
  Artificial Sequence-LCDR3 of 14C12
LQYDEFPLT

SEQ ID NO: 33 - protein, 8 aa, Artificial Sequence
  Artificial Sequence-HCDR1 of 4G10
GYSFTGYT

SEQ ID NO: 34 - protein, 8 aa, Artificial Sequence
  Artificial Sequence-HCDR2 of 4G10
INPYNNIT

SEQ ID NO: 35 - protein, 8 aa, Artificial Sequence
  Artificial Sequence-HCDR3 of 4G10
ARLDYRSY

SEQ ID NO: 36 - protein, 9 aa, Artificial Sequence
  Artificial Sequence-LCDR1 of 4G10
TGAVTTSNF

SEQ ID NO: 37 - protein, 3 aa, Artificial Sequence
  Artificial Sequence-LCDR2 of 4G10
GTN

SEQ ID NO: 38 - protein, 9 aa, Artificial Sequence
  Artificial Sequence-LCDR3 of 4G10
ALWYSNHWV

SEQ ID NO: 39 - DNA, 1344 bp, Artificial Sequence
  Artificial Sequence-DNA sequence of heavy chain of immunoglobulin moiety of CP004(hG1TM)
gaagtgcagctggtcgagtctgggggagggctggtgcagcccggcgggtcactgcgactgagctgcgcagcttccggattcgcctttagctcctacgacatgtcctgggtgcgacaggcaccaggaaagggactggattgggtcgctactatctcaggaggcgggagatacacctactatcctgacagcgtcaagggccggttcacaatctctagagataacagtaagaacaatctgtatctgcagatgaacagcctgagggctgaggacaccgcactgtactattgtgccaaccgctacggggaagcatggtttgcctattgggggcagggaaccctggtgacagtctctagtgccagcaccaaagggcccagcgtgtttcctctcgccccctcctccaaaagcaccagcggaggaaccgctgctctcggatgtctggtgaaggactacttccctgaacccgtcaccgtgagctggaatagcggcgctctgacaagcggagtccatacattccctgctgtgctgcaaagcagcggactctattccctgtccagcgtcgtcacagtgcccagcagcagcctgggcacccagacctacatctgtaacgtcaaccacaagccctccaacaccaaggtggacaagaaagtggagcccaaatcctgcgacaagacacacacctgtcccccctgtcctgctcccgaagctgctggagcccctagcgtcttcctctttcctcccaaacccaaggacaccctcatgatcagcagaacccctgaagtcacctgtgtcgtcgtggatgtcagccatgaggaccccgaggtgaaattcaactggtatgtcgatggcgtcgaggtgcacaacgccaaaaccaagcccagggaggaacagtacaactccacctacagggtggtgtccgtgctgacagtcctccaccaggactggctgaacggcaaggagtacaagtgcaaggtgtccaacaaggctctccctgcccccattgagaagaccatcagcaaggccaaaggccaacccagggagccccaggtctatacactgcctccctccagggacgaactcaccaagaaccaggtgtccctgacctgcctggtcaagggcttttatcccagcgacatcgccgtcgagtgggagtccaacggacagcccgagaataactacaagaccacccctcctgtcctcgactccgacggctccttcttcctgtacagcaagctgaccgtggacaaaagcaggtggcagcagggaaacgtgttctcctgcagcgtgatgcacgaagccctccacaaccactacacccagaaaagcctgtccctgagccccggcaaa

SEQ ID NO: 40 - protein, 448 aa, Artificial Sequence
  Artificial Sequence-amino acid sequence of heavy chain of immunoglobulin moiety in CP004(hG1TM)
EVQLVESGGGLVQPGGSLRLSCAASGFAFSSYDMSWVRQAPGKGLDWVATISGGGRYTYYPDSVKGRFTISRDNSKNNLYLQMNSLRAEDTALYYCANRYGEAWFAYWGQGTLVTVSSASTKGPSVFPLAPSSKSTSGGTAALGCLVKDYFPEPVTVSWNSGALTSGVHTFPAVLQSSGLYSLSSVVTVPSSSLGTQTYICNVNHKPSNTKVDKKVEPKSCDKTHTCPPCPAPEAAGAPSVFLFPPKPKDTLMISRTPEVTCVVVDVSHEDPEVKFNWYVDGVEVHNAKTKPREEQYNSTYRVVSVLTVLHQDWLNGKEYKCKVSNKALPAPIEKTISKAKGQPREPQVYTLPPSRDELTKNQVSLTCLVKGFYPSDIAVEWESNGQPENNYKTTPPVLDSDGSFFLYSKLTVDKSRWQQGNVFSCSVMHEALHNHYTQKSLSLSPGK

SEQ ID NO: 41 - protein, 115 aa, Artificial Sequence
  Artificial Sequence-amino acid sequence of 4G10H1V(M)
QVQLVESGAELVKPGASMKISCKASGYSFTGYTMNWVKQAPGQCLEWIGLINPYNNITNYNQKFMGKATFTVDKSISTAYMELSRLTSDDSGVYFCARLDYRSYWGQGTLVTVSA

SEQ ID NO: 42 - protein, 110 aa, Artificial Sequence
  Artificial Sequence-amino acid sequence of 4G10L1V(M)
QAVVTQEPSLTVSPGGTVTLTCGSSTGAVTTSNFANWVQEKPGQAFRSLIGGTNNRASWVPARFSGSLLGGKAALTISGAQPEDEAEYFCALWYSNHWVFGCGTKLTVLR

SEQ ID NO: 43 - protein, 115 aa, Artificial Sequence
  Artificial Sequence-amino acid sequence of 4G10H3V(M)
QVQLVESGAEVKKPGASVKVSCKASGYSFTGYTMNWVRQAPGQCLEWIGLINPYNNITNYAQKFQGRVTFTVDTSISTAYMELSRLRSDDTGVYFCARLDYRSYWGQGTLVTVSA

SEQ ID NO: 44 - protein, 110 aa, Artificial Sequence
  Artificial Sequence-amino acid sequence of 4G10L3V(M)
QAVVTQEPSLTVSPGGTVTLTCGSSTGAVTTSNFPNWVQQKPGQAPRSLIGGTNNKASWTPARFSGSLLGGKAALTISGAQPEDEAEYYCALWYSNHWVFGCGTKLTVLR

SEQ ID NO: 45 - protein, 116 aa, Artificial Sequence
  Artificial Sequence-sequence of heavy chain variable region of hIgG
EVQLEQSGAELMKPGASVKISCKATGYTFTTYWIEWIKQRPGHSLEWIGEILPGSDSTYYNEKVKGKVTFTADASSNTAYMQLSSLTSEDSAVYYCARGDGFYVYWGQGTTLTVSS

SEQ ID NO: 46 - protein, 327 aa, Artificial Sequence
  Artificial Sequence-sequence of heavy chain constant region of hIgG
ASTKGPSVFPLAPCSRSTSESTAALGCLVKDYFPEPVTVSWNSGALTSGVHTFPAVLQSSGLYSLSSVVTVPSSSLGTKTYTCNVDHKPSNTKVDKRVESKYGPPCPPCPAPEFLGGPSVFLFPPKPKDTLMISRTPEVTCVVVDVSQEDPEVQFNWYVDGVEVHNAKTKPREEQFNSTYRVVSVLTVLHQDWLNGKEYKCKVSNKGLPSSIEKTISKAKGQPREPQVYTLPPSQEEMTKNQVSLTCLVKGFYPSDIAVEWESNGQPENNYKTTPPVLDSDGSFFLYSRLTVDKSRWQEGNVFSCSVMHEALHNHYTQKSLSLSLGK

SEQ ID NO: 47 - protein, 107 aa, Artificial Sequence
  Artificial Sequence-sequence of light chain variable region of hIgG
DIELTQSPATLSVTPGDSVSLSCRASQSISNNLHWYQQKSHESPRLLIKYTSQSMSGIPSRFSGSGSGTDFTLSINSVETEDFGVYFCQQSGSWPRTFGGGTKLDIK

SEQ ID NO: 48 - protein, 107 aa, Artificial Sequence [sequence omitted]

SEQ ID NO: 49 - DNA, 348 bp, Artificial Sequence
  Artificial Sequence-nucleic acid sequence of heavy chain variable region of HpL3
gaagtgcagctggtgcagagcggcgggggactggtgaagcccggcgggtccctgcgactgtcttgcgccgctagtggcttcaccttcagctcctactctatgaactgggtgagacaggcccctggaaaaggcctggagtgggtctctagtatctcaagctcctctagttacatctactatgccgacagcgtgaaggggcggttcaccatctcaagagataacgctaaaaatagtctgtatctgcagatgaacagcctgagggcagaagacactgccgtgtactattgtgctcgcgtcaccgacgcatttgatatttgggggcagggaaccatggtgacagtctcaagc

SEQ ID NO: 50 - protein, 116 aa, Artificial Sequence [sequence omitted]

SEQ ID NO: 51 - DNA, 321 bp, Artificial Sequence
  Artificial Sequence-nucleic acid sequence of light chain variable region of HpL3
gacattcagatgactcagagcccttcttcagtgtccgcctctatcggcgaccgggtcaccattacatgcagagcttcccagggcctcgataactggctggggtggtaccagcagaagcctgggaaagccccaaagctgctgatctacgacgcttccaatctggataccggagtgccatctcgattcagtggctcagggagcggaacatactttactctgaccatcagctccctgcaggctgaggacttcgcagtgtatttttgccagcaggcaaaggccttccctcccacctttggcgggggaacaaaagtggacatcaag

SEQ ID NO: 52 - protein, 107 aa, Artificial Sequence
  Artificial Sequence-amino acid sequence of light chain variable region of HpL3
DIQMTQSPSSVSASIGDRVTITCRASQGLDNWLGWYQQKPGKAPKLLIYDASNLDTGVPSRFSGSGSGTYFTLTISSLQAEDFAVYFCQQAKAFPPTFGGGTKVDIK

SEQ ID NO: 53 - protein, 8 aa, Artificial Sequence
  Artificial Sequence-HCDR1 of heavy chain variable region of HpL3
GFTFSSYS

SEQ ID NO: 54 - protein, 8 aa, Artificial Sequence
  Artificial Sequence-HCDR2 of heavy chain variable region of HpL3
ISSSSSYI

SEQ ID NO: 55 - protein, 9 aa, Artificial Sequence
  Artificial Sequence-HCDR3 of heavy chain variable region
ARVTDAFDI

SEQ ID NO: 56 - protein, 6 aa, Artificial Sequence
  Artificial Sequence-LCDR1 of light chain variable region of HpL3
QGLDNW

SEQ ID NO: 57 - protein, 3 aa, Artificial Sequence
  Artificial Sequence-LCDR2 of light chain variable region
DAS

SEQ ID NO: 58 - protein, 9 aa, Artificial Sequence
  Artificial Sequence-LCDR3 of light chain variable region of HpL3
QQAKAFPPT

SEQ ID NO: 59 - DNA, 369 bp, Artificial Sequence
  Artificial Sequence-nucleic acid sequence of heavy chain variable region of bevacizumab
gaggtgcagctggtcgagtccgggggggggctggtgcagccaggcgggtctctgaggctgagttgcgccgcttcagggtacaccttcacaaactatggaatgaattgggtgcgccaggcaccaggaaagggactggagtgggtcggctggatcaacacttacaccggggaacctacctatgcagccgactttaagcggcggttcaccttcagcctggatacaagcaaatccactgcctacctgcagatgaacagcctgcgagctgaggacaccgcagtctactattgtgctaaatatccccactactatgggagcagccattggtattttgacgtgtgggggcaggggactctggtgacagtgagcagc

SEQ ID NO: 60 - protein, 123 aa, Artificial Sequence [sequence omitted]

SEQ ID NO: 61 - DNA, 321 bp, Artificial Sequence
  Artificial Sequence-nucleic acid sequence of light chain variable region of bevacizumab
gatattcagatgactcagagcccctcctccctgtccgcctctgtgggcgacagggtcaccatcacatgcagtgcttcacaggatatttccaactacctgaattggtatcagcagaagccaggaaaagcacccaaggtgctgatctacttcactagctccctgcactcaggagtgccaagccggttcagcggatccggatctggaaccgactttactctgaccatttctagtctgcagcctgaggatttcgctacatactattgccagcagtattctaccgtgccatggacatttggccaggggactaaagtcgagatcaag

SEQ ID NO: 62 - protein, 107 aa, Artificial Sequence [sequence omitted]

SEQ ID NO: 63 - protein, 8 aa, Artificial Sequence
  Artificial Sequence-HCDR1 of heavy chain variable region of bevacizumab
GYTFTNYG

SEQ ID NO: 64 - protein, 8 aa, Artificial Sequence
  Artificial Sequence-HCDR2 of heavy chain variable region of bevacizumab
INTYTGEP

SEQ ID NO: 65 - protein, 16 aa, Artificial Sequence
  Artificial Sequence-HCDR3 of heavy chain variable region of bevacizumab
AKYPHYYGSSHWYFDV

SEQ ID NO: 66 - protein, 6 aa, Artificial Sequence
  Artificial Sequence-LCDR1 of light chain variable region of bevacizumab
QDISNY

SEQ ID NO: 67 - protein, 3 aa, Artificial Sequence
  Artificial Sequence-LCDR2 of light chain variable region of bevacizumab
FTS

SEQ ID NO: 68 - protein, 9 aa, Artificial Sequence
  Artificial Sequence-LCDR3 of light chain variable region of bevacizumab
QQYSTVPWT

SEQ ID NO: 69 - DNA, 2139 bp, Artificial Sequence
  Artificial Sequence-nucleic acid sequence of CP004(hG1TM) heavy chain
gaagtgcagctggtcgagtctgggggagggctggtgcagcccggcgggtcactgcgactgagctgcgcagcttccggattcgcctttagctcctacgacatgtcctgggtgcgacaggcaccaggaaagggactggattgggtcgctactatctcaggaggcgggagatacacctactatcctgacagcgtcaagggccggttcacaatctctagagataacagtaagaacaatctgtatctgcagatgaacagcctgagggctgaggacaccgcactgtactattgtgccaaccgctacggggaagcatggtttgcctattgggggcagggaaccctggtgacagtctctagtgccagcaccaaagggcccagcgtgtttcctctcgccccctcctccaaaagcaccagcggaggaaccgctgctctcggatgtctggtgaaggactacttccctgaacccgtcaccgtgagctggaatagcggcgctctgacaagcggagtccatacattccctgctgtgctgcaaagcagcggactctattccctgtccagcgtcgtcacagtgcccagcagcagcctgggcacccagacctacatctgtaacgtcaaccacaagccctccaacaccaaggtggacaagaaagtggagcccaaatcctgcgacaagacacacacctgtcccccctgtcctgctcccgaagctgctggagcccctagcgtcttcctctttcctcccaaacccaaggacaccctcatgatcagcagaacccctgaagtcacctgtgtcgtcgtggatgtcagccatgaggaccccgaggtgaaattcaactggtatgtcgatggcgtcgaggtgcacaacgccaaaaccaagcccagggaggaacagtacaactccacctacagggtggtgtccgtgctgacagtcctccaccaggactggctgaacggcaaggagtacaagtgcaaggtgtccaacaaggctctccctgcccccattgagaagaccatcagcaaggccaaaggccaacccagggagccccaggtctatacactgcctccctccagggacgaactcaccaagaaccaggtgtccctgacctgcctggtcaagggcttttatcccagcgacatcgccgtcgagtgggagtccaacggacagcccgagaataactacaagaccacccctcctgtcctcgactccgacggctccttcttcctgtacagcaaactgaccgtggataagtccagatggcagcagggcaatgtcttttcatgttccgtgatgcacgaggcactgcacaaccactatacccagaagtctctgagtctgtcaccaggaaaaggaggaggaggctctggaggaggcggaagtggaggcggaggatcaggagggggaggatctcaggtgcagctggtcgaatccggagccgaggtgaagaaacccggcgcttccgtgaaggtctcttgcaaagcatcaggctacagcttcacagggtatactatgaactgggtgcggcaggcacctggacagtgtctggaatggatcggcctgattaacccatacaacaacatcactaactacgcccagaagttccagggccgggtgacttttaccgtggacactagcatttccaccgcttacatggagctgagtcggctgagatcagacgataccggcgtgtatttttgcgcaaggctggattacagaagttattggggacagggaacacttgttacagtctctgctggaggaggcggatctggaggaggaggatctggcggaggaggcagtggaggaggaggatcacaggctgtggttactcaggaaccaagcctgaccgtgagccccggaggcacagtcactctgacctgtgggagctccacaggagctgtgaccacatctaacttccctaattgggtgcagcagaagccaggacaggcacctcgatccctgatcgggggaaccaacaacaaggccagctggacacccgccagattttctggcagtctgctgggcgggaaagccgctctgaccattagcggcgctcagcctgaggacgaagcagagtactattgcgccctgtggtatagtaatcattgggtgttcgggtgtgggacaaaactgaccgtgctgaga

SEQ ID NO: 70 - protein, 713 aa, Artificial Sequence
  Artificial Sequence-amino acid sequence of CP004(hG1TM) heavy chain
EVQLVESGGGLVQPGGSLRLSCAASGFAFSSYDMSWVRQAPGKGLDWVATISGGGRYTYYPDSVKGRFTISRDNSKNNLYLQMNSLRAEDTALYYCANRYGEAWFAYWGQGTLVTVSSASTKGPSVFPLAPSSKSTSGGTAALGCLVKDYFPEPVTVSWNSGALTSGVHTFPAVLQSSGLYSLSSVVTVPSSSLGTQTYICNVNHKPSNTKVDKKVEPKSCDKTHTCPPCPAPEAAGAPSVFLFPPKPKDTLMISRTPEVTCVVVDVSHEDPEVKFNWYVDGVEVHNAKTKPREEQYNSTYRVVSVLTVLHQDWLNGKEYKCKVSNKALPAPIEKTISKAKGQPREPQVYTLPPSRDELTKNQVSLTCLVKGFYPSDIAVEWESNGQPENNYKTTPPVLDSDGSFFLYSKLTVDKSRWQQGNVFSCSVMHEALHNHYTQKSLSLSPGKGGGGSGGGGSGGGGSGGGGSQVQLVESGAEVKKPGASVKVSCKASGYSFTGYTMNWVRQAPGQCLEWIGLINPYNNITNYAQKFQGRVTFTVDTSISTAYMELSRLRSDDTGVYFCARLDYRSYWGQGTLVTVSAGGGGSGGGGSGGGGSGGGGSQAVVTQEPSLTVSPGGTVTLTCGSSTGAVTTSNFPNWVQQKPGQAPRSLIGGTNNKASWTPARFSGSLLGGKAALTISGAQPEDEAEYYCALWYSNHWVFGCGTKLTVLR

SEQ ID NO: 71 - DNA, 642 bp, Artificial Sequence; identical to SEQ ID NO: 23
  Artificial Sequence-nucleic acid sequence of CP004(hG1TM) light chain

SEQ ID NO: 72 - protein, 214 aa, Artificial Sequence; identical to SEQ ID NO: 24
  Artificial Sequence-amino acid sequence of CP004(hG1TM) light chain